European Patent Application EP 4 230 221 A1, published August 23, 2023. Title: Pharmaceutical composition for preventing or treating retinal or choroidal disease comprising PLVAP as an active ingredient. Applicant: THE ASAN FOUNDATION University of Ulsan Foundation For Industry Cooperation. The sequence listing filed with the application follows.

SEQUENCE LISTING (25 sequences)

SEQ ID NO: 1 - DNA, 1329 bp, Artificial Sequence
  hPLVAP
atgggtctggccatggagcacggagggtcctacgctcgggcggggggcagctctcggggctgctggtattacctgcgctacttcttcctcttcgtctccctcatccaattcctcatcatcctggggctcgtgctcttcatggtctatggcaacgtgcacgtgagcacagagtccaacctgcaggccaccgagcgccgagccgagggcctatacagtcagctcctagggctcacggcctcccagtccaacttgaccaaggagctcaacttcaccacccgcgccaaggatgccatcatgcagatgtggctgaatgctcgccgcgacctggaccgcatcaatgccagcttccgccagtgccagggtgaccgggtcatctacacgaacaatcagaggtacatggctgccatcatcttgagtgagaagcaatgcagagatcaattcaaggacatgaacaagagctgcgatgccttgctcttcatgctgaatcagaaggtgaagacgctggaggtggagatagccaaggagaagaccatttgcactaaggataaggaaagcgtgctgctgaacaaacgcgtggcggaggaacagctggttgaatgcgtgaaaacccgggagctgcagcaccaagagcgccagctggccaaggagcaactgcaaaaggtgcaagccctctgcctgcccctggacaaggacaagtttgagatggaccttcgtaacctgtggagggactccattatcccacgcagcctggacaacctgggttacaacctctaccatcccctgggctcggaattggcctccatccgcagagcctgcgaccacatgcccagcctcatgagctccaaggtggaggagctggcccggagcctccgggcggatatcgaacgcgtggcccgcgagaactcagacctccaacgccagaagctggaagcccagcagggcctgcgggccagtcaggaggcgaaacagaaggtggagaaggaggctcaggcccgggaggccaagctccaagctgaatgctcccggcagacccagctagcgctggaggagaaggcggtgctgcggaaggaacgagacaacctggccaaggagctggaagagaagaagagggaggcggagcagctcaggatggagctggccatcagaaactcagccctggacacctgcatcaagaccaagtcgcagccgatgatgccagtgtcaaggcccatgggccctgtccccaacccccagcccatcgacccagctagcctggaggagttcaagaggaagatcctggagtcccagaggccccctgcaggcatccctgtagccccatccagtggctga

SEQ ID NO: 2 - DNA, 1317 bp, Artificial Sequence
  mPLVAP
atggggctctccatggaccgcagcccatacgcccgcacgggggaccagcagcgcggctgctggtactacctgcgctatttcttcctcttcgtgtcgctcattcagttcctcatcatcctgggcctggtcctcttcatgatctatggcaatgtgcacgccaccactgagtccagcctgcgcgccacggagatccgcgccgacagcctgtacagccaggtggttggactatcggcctcacaggctaacctgagcaaacagctgaacatcagcttgcttgtcaaggaaacagtcatgcagcaactgttgactacgcgacgtgagatggagcgcatcaacgccagcttccgccagtgccaaggcgacctgatcacctacataaactataatcgcttcatcgccgctatcatcctgagcgagaagcagtgccaggaacagctgaaggaggtcaacaagacctgcgaagctttactcttcaagctgggagaaaaagttaagacactggagatggaggtggccaaggagaaggcagtgtgctccaaggacaaggagagcctgctggcaggaaagcggcagacggaagagcagctggaggcctgtggcaaagcacgcgaaaggcaacagcaggagcagcaggtgaccgaggagaacctgcgcaaggtgcagtccctgtgcatcccactggaccaggagaagttccaggcggacgtgctgagtgcgtggcgggactcgctgatctaccgtaccttggaaaccctgccctaccactaccagctgatgccggagtacgcgtccctccgtcggacctgcgagagcctgcccgggatcatgaccaccaagatagaagagctggcccgcgggctgcgcgccggcattgagcgcgtgacccgtgagaatgcagaactgcggcgccagaagttggagctagagcgcgcggcacaggcggcgcaggaggcgcgggcgcgcgccgggaccgaggcgcaggcgcgagaaacccagctacgggcggagtgcgcgcgccagacgcagctggctctggaggagaaggcggcgctgcgcgcgcagcgggacaacctagagcgcgagctggaggcgcgtaagcgggagctggagcaactgcgcaccgaggtggatgtgcgcattagcgcgctggacacctgcgtcaaggccaagtcgctgccagccgtcccgccgagagtctcaggcccacccccgaaccctccacccattgatccagctagcctggaggaattcaagaaaaggatcctggagtctcagcggctccctgtagtcaaccctgctgcccaacccagcggttga

SEQ ID NO: 3 - DNA, 584 bp, Artificial Sequence
  h/mCMV
gacattgattattgactagttattaatagtaatcaattacggggtcattagttcatagcccatatatggagttccgcgttacataacttacggtaaatggcccgcctggctgaccgcccaacgacccccgcccattgacgtcaataatgacgtatgttcccatagtaacgccaatagggactttccattgacgtcaatgggtggagtatttacggtaaactgcccacttggcagtacatcaagtgtatcatatgccaagtacgccccctattgacgtcaatgacggtaaatggcccgcctggcattatgcccagtacatgaccttatgggactttcctacttggcagtacatctacgtattagtcatcgctattaccatggtgatgcggttttggcagtacatcaatgggcgtggatagcggtttgactcacggggatttccaagtctccaccccattgacgtcaatgggagtttgttttggcaccaaaatcaacgggactttccaaaatgtcgtaacaactccgccccattgacgcaaatgggcggtaggcgtgtacggtgggaggtctatataagcagagct

SEQ ID NO: 4 - DNA, 1559 bp, Artificial Sequence
  hCD144
catccatgcccatggcctcagatgccagccataagctgttgggttccaaacctcgactccaggctggactcacccctgtctcccccaccagcctgacacctccacctgggtatctaacgagcatctcaaactcaacctgcctgagacagaggaatcactatcccctcctcctccaaaaatatccttccatcacactccccatcttgtgctctgatttactaaacggccctgggccctctctttctcagggtctctgcttgcccagctatataataaaacaagtttgggacttcccaaccattcacccatggaaaaacagaagcaactcttcaaaggacagattcccaggatctgccctgggagattccaaatcagttgatctggggtgagcccagtcctctgtagtttttagaagctcctcctatgtctctcctggtcagcagaatcttggcccctcccttccccccagcctcttggttcttctgggctctgatccagcctcagcgtcactgtcttccacgcccctctttgattctcgtttatgtcaaaagccttgtgaggatgaggctgtgattatccccattttacagatgaggaaactgtggctccaggatgacacaactggccagaggtcacatcagaagcagagctgggtcacttgactccacccaatatccctaaatgcaaacatcccctacagaccgaggctggcaccttagagctggagtccatgcccgctctgaccaggagaagccaacctggtcctccagagccaagagcttctgtccctttcccatctcctgaagcctccctgtcacctttaaagtccattcccacaaagacatcatgggatcaccacagaaaatcaagctctggggctaggctgaccccagctagatttttggctcttttataccccagctgggtggacaagcaccttaaacccgctgagcctcagcttcccgggctataaaatgggggtgatgacacctgcctgtagcattccaaggagggttaaatgtgatgctgcagccaagggtccccacagccaggctctttgcaggtgctgggttcagagtcccagagctgaggccgggagtaggggttcaagtggggtgccccaggcagggtccagtgccagccctctgtggagacagccatccggggccgaggcagccgcccaccgcagggcctgcctatctgcagccagcccagccctcacaaaggaacaataacaggaaaccatcccagggggaagtgggccagggccagctggaaaacctgaaggggaggcagccaggcctccctcgccagcggggtgtggctcccctccaaagacggtcggctgacaggctccacagagctccactcacgctcagccctggacggacaggcagtccaacggaacagaaacatccctcagcccacaggcacggtgagtgggggctcccacactcccctccaccccaaacccgccaccctgcgcccaagatgggagggtcctcagcttccccatctgtagaatgggcatcgtcccactcccatgacagagaggctcc

SEQ ID NO: 5 - DNA, 2510 bp, Artificial Sequence
  mCD144
ctagtagcagaaacaaggtcctctggaagagcaactgatgctcttaggtactgaagcatcatcctgccccagagaccactcgcatatgaagcacacatattcagtctgccttacttgtgttaatgattgccagtgtccctctgacctcctagccctgaaaagtgtggcctgaaggtcatttcagagacggggagagctgctcagagaagccaatcggcgagtctaggacacacagacaggatctagtcccagagttcgctagcctaggtgagcgtcccctggccccttataccacttccttctccagcttgcatctaatctgctctggcagaccatcgtgtttcctgtcttcctggcagcctccagcacgctcagtgctactccctgcgcatgcgccctcctcccagtaccttctctgactccagtgggcttggagtgcgaggaggaagggtgaggaaggggtgaaatcaggtattggatccacagggggtctgaagagcactagcctggccttttgggactgaacttctgctatgaagacctccactgccatccctggagtccggggcacatccaaggcttgctgtccatcgtttactgtttacagatgacaacaatgactgtgttcggggcagaaatatccaccagggctagagtacaaaaggagtttgcattgatggccggacaggccctgtccctggcagcctgccagcgctgagtatgagacccagcgggaagtgctaccctggcagacgtgtccactgagtacacagaccaccaaggcaggcagctctcggggaagctgtctatgctgggccagcccaccttgagggcagggaacagaacagattgtggcagagaggaaaatgtggagcttctgtttgttcacagacacacgcactcgcccacgcacgcacgcacgcacgcacgcacgcacgaatgcacgcacgcagtagttgaatgctatggattccgctcagagctgagaacagccccagcgacagttccctggcctctctccttactctgatgtcctcatctgtcttcacatggtctcaggacgctaatactccatcctaatgtacactcctttccctgggcctccgttccagttcagttctcagaggacctggagggagtgattggctacaccaactttgctttcgttcaccaagcccatgtctctacttgggtgtctaatgggcatctccaacattacctaccccaaacagaaaaccctttcttccccccaaccacaccccaccctacccccacagtattttctccatgcccggaaagatctgctctcttatggtccctctttgcctcactgaaaagcaggacaagttggggacttcccaaacttttatgcatgaagaaacccaggcaatttgccaaaaggtacactctgggggtctgtcatttactctgagccagaaccctgaaatttttactaacccatcacataatgaatgaagagaatctttttctttttttttttttttctttttttttggtttttcgagacagggtttctctgtatagccctggctatcctggaacacactctgtagaccaggctggcctcgaactcagaaatccacctgcctctgcctcccgagtgctgggattaaaggcgtgcgccaccacgcctggctgaatgaagagaatcttgacctcatctccccagcctcttggtcctgagggaccctggtctacctactgctttgctgtcttcttagctcttcttacttttttgctgactcagacctatggctatctccattatacagatgaggagactgaggcatggatccctggttggtccatggtcacgtgaagcccatcacccagtatttgtaaagtgagatgggccaggctggtaccttggaactgaaactcacactgccctacctggaagaatctgacaggcaaaatctgctgctgaaagtgattgtctgtcacgtttctcagctgcccgactctgagaactccacagccccctttcgttccaccatactacagagtcgccacggaaagccggctctgtggagaagctgaggtagctgggtttctgtctgggttactctgtccagcgaggaaacaagtaccttagacccactaagcctctgctttctgaactgtaaagtgggggatatgacacctgcctcccagggatggctgaatgctctggcagaagcttagagcccccacagctacccctaggctcacagctcctccgatgagacctagaattgaggtatgagttgaataccccaggcaggtccaaggcttccacgggcccaggctgaccaagctgaggccgcccaccgtagggcttgcctatctgcaggcagctcacaaaggaacaataacaggaaaccatcccgaggggaagtgggccagggccagttggaaaacctgcctccctcccagcctgggtgtggctcccctctcccctcctgaggcaatcaactgtgctctccacaaagctcggccctggacagact

SEQ ID NO: 6 - DNA, 2527 bp, Artificial Sequence
  hTIE1
atttcctcttcctccccagcaccgacccacactgaccaacacaggctgagcagtcaggcccacagcatctgaccccaggcccagctcgtcctggctggcctgggtcggcctctggagtatggtctggcgggtgccccctttcttgctccccatcctcttcttggcttctcatgtgggcgcggcggtggacctgacgctgctggccaacctgcggctcacggacccccagcgcttcttcctgacttgcgtgtctggggaggccggggcggggaggggctcggacgcctggggcccgcccctgctgctggagaaggacgaccgtatcgtgcgcaccccgcccgggccacccctgcgcctggcgcgcaacggttcgcaccaggtcacgcttcgcggcttctccaagccctcggacctcgtgggcgtcttctcctgcgtgggcggtgctggggcgcggcgcacgcgcgtcatctacgtgcacaacagccctggagcccacctgcttccagacaaggtcacacacactgtgaacaaaggtgacaccgctgtactttctgcacgtgtgcacaaggagaagcagacagacgtgatctggaagagcaacggatcctacttctacaccctggactggcatgaagcccaggatgggcggttcctgctgcagctcccaaatgtgcagccaccatcgagcggcatctacagtgccacttacctggaagccagccccctgggcagcgccttctttcggctcatcgtgcggggttgtggggctgggcgctgggggccaggctgtaccaaggagtgcccaggttgcctacatggaggtgtctgccacgaccatgacggcgaatgtgtatgcccccctggcttcactggcacccgctgtgaacaggcctgcagagagggccgttttgggcagagctgccaggagcagtgcccaggcatatcaggctgccggggcctcaccttctgcctcccagacccctatggctgctcttgtggatctggctggagaggaagccagtgccaagaagaccggatcccccagatcctcaacatggcctcagaactggagttcaacttagagacgatgccccggatcaactgtgcagctgcagggaaccccttccccgtgcggggcagcatagagctacgcaagccagacggcactgtgctcctgtccaccaaggccattgtggagccagagaagaccacagctgagttcgaggtgccccgcttggttcttgcggacagtgggttctgggagtgccgtgtgtccacatctggcggccaagacagccggcgcttcaaggtcaatgtgaaagtgccccccgtgcccctggctgcacctcggctcctgaccaagcagagccgccagcttgtggtctccccgctggtctcgttctctggggatggacccatctccactgtccgcctgcactaccggccccaggacagtaccatggactggtcgaccattgtggtggaccccagtgagaacgtgacgttaatgaacctgaggccaaagacaggatacagtgttcgtgtgcagctgagccggccaggggaaggaggagagggggcctgggggcctcccaccctcatgaccacagactgtcctgagcctttgttgcagccgtggttggagggctggcatgtggaaggcactgaccggctgcgagtgagctggtccttgcccttggtgcccgggccactggtgggcgacggtttcctgctgcgcctgtgggacgggacacgggggcaggagcggcgggagaacgtctcatccccccaggcccgcactgccctcctgacgggactcacgcctggcacccactaccagctggatgtgcagctctaccactgcaccctcctgggcccggcctcgccccctgcacacgtgcttctgccccccagtgggcctccagccccccgacacctccacgcccaggccctctcagactccgagatccagctgacatggaagcacccggaggctctgcctgggccaatatccaagtacgttgtggaggtgcaggtggctgggggtgcaggagacccactgtggatagacgtggacaggcctgaggagacaagcaccatcatccgtggcctcaacgccagcacgcgctacctcttccgcatgcgggccagcattcaggggctcggggactggagcaacacagtagaagagtccaccctgggcaacgggctgcaggctgagggcccagtccaagagagccgggcagctgaagagggcctggatcagcagctgatcctggcggtggtgggctccgtgtctgccacctgcctcaccatcctggctgcccttttaaccctggtgtgcatccgcagaagctgcctgcatcggagacgcaccttcacctaccagtcaggctcgggcgaggagaccatcctgcagttcagctcagggaccttgacacttacccggcggccaaaactgcagcccgagcccctgagctacccagtgctagagtgggaggacatcacctttgaggacctcatcggg

SEQ ID NO: 7 - DNA, 1063 bp, Artificial Sequence
  mTIE1
aaaagaaaaagaaaaacctgcagaagtatgtgccagcagactggaagctaagggaagaggagcctgggcttggacaacctggctctgctcccttctaactgtatgaccttaggcaagttttgagcttttgctccctggttataaaaccatcatcctggaagaggataacactcacctcccaggacagtgtggtcctgaaaggacgagagcatcactaaagggccccggcacataattgacatccaataaacattaattattatgacagcaggaacacaagatgactctgaagttagtgtctcaggtaatgggtgttatcctttgactcagaaagcttgggagaggtgagggtgtagcttaggaaacacagatgcaaatgcattgggagctgaaaggccacaccagagctactgactcaggggtgacagttaatgccgagggagtggatgaatgtgctccgtagttattacagcaaaggatgtcaacttcactggaagccatgaggatgccagggagaaagggcatttggtgcccgcgaggtggccaagagatgccagcttctttggcttacgatagaccgtcaaaaatatgctaagtggcatttaaatgaattgatgacctgacagctaacaggcagggaagggccagggaaggaggggccttggaaggtctggggtcacaggtctgaagcaggctgatcacattcttctcctcggtcttgcccacttcagggtacagattttacgctccagttgcactagcccggggcagctcccctccccacactacaacatttctcatacttgagcgtagggtggcctctccctacgcctgacctttcgttcctcctcacccaagcaccttctaatgaagtttgttatctgcatcttttcctgtcccctttccttcccccgcccccctgctggttagatgttcctccctctgagccaacacctccatctgggagggatgcctgtgtctggtcctccagcttcccaaggtagggcccagacccacctgtgtctgtgtctctctggccctaaccgatcttcaatcccagcca

SEQ ID NO: 8 - DNA, 1234 bp, Artificial Sequence
  hFLT1
gtttaagcaatttggtagaaccgaacagtccattctgctccattggccttcgtttataggagaggcttgtaagaaatgacaagatctcctgccagatgctttccaggatcactggtggttcctcacactcttgggtgctgtggaaattgcatgctgctgattaaattgctggattttataccagattgagggaggggaaggaaattggaggaatggggtatttgagggagggcttgaaaagaaagcctctgacttagctcacggggctgcaggggggttcattaaggaaacagttgcattgagtctgctgaagatagtggactagatttcctgcattgccgctggggcggatgtggggagatgtcaagaattcctggggatttcccatccatcttggtaaagctggatgcctgaaagctgtttctgattgctgctcctttcctcaattttgagctctttgaggaacttgatcttgtctcacagatacacacacacgttgtaagagctagatggaacctcattgacccaatctactcatgccagagatgagaaaaccggcccagaggaggccagtgctgtttttcaaggtcaacagctggctagcggcaggcctaggaacagaacctgatgttcctgctacagacaacatctcttcttcactggtgtatttcctcttccccagacggaagacagatgttcaaatatttattgactaacattattacagtgctaaaatttctttcgaaatgacatctttttaatatgaagttttcttctattttcttaacgcacataaggggtttaaactaagaatcaaaatgatggctgcttagtagcatgccaagagatttgatgagaagattaactttccttacgagcacttggtatccttttcctgaacagctgtggcttacatacttgtggcttatggtactagctttgtctttcgccacttctctccacacacacactgggttccagctacacaaactctaccctagtcaaacaaattattcccccttcttcagaggcgccttcactttcatcactctgttcatgctgctcgtctgcctgcaagaccttttccctccctctgtgtctcctcctctcctgctggcaagatccagcccagtaatcaccatctctgggagctcctccttgtagctcccagacagcacttgccatttcttctgctctcctgtagccctgaggtgtactcctccttcagtaattc

SEQ ID NO: 9 - DNA, 1360 bp, Artificial Sequence
  mFLT1
tggtcccatttaggagccattttatcacgggtatctggcaggttctattgaggctatttttcaaacctgcagtatttacagggacaagactgggctgctccggggaggccgggacgacttcagccttccagttaatggatgcataattgaggaacaacgtggaattagtgtcatcgtaaatgatctagtgtctcaagttaatttcacccgttttttgttccaagaacattcgagtcagtcatcttggctagccggcttccaccaaaaagatttgttttccatccagcgtttcagacctagagttcaagttcttggcccttacaagttgcaggagcgtgtctcacgccttggcttttttttttttttttttttttttttttaaggtaacatgttattccttgttttgcttctaggaagcagagggttgaggaaatggcttgggcgggtgcattaatgcagccgaaaaagacacagactccctcccttgggacccgcgcggccccgcgctctttccgaaggtgcctggcaaggcgtccggttccctcggacgctccgggtccaagtgccttaagcggagggtctctggcgccttccttcgctgtctggcaacagtctggcggggtcagggaccggcgggaccgctcgggagagggctcgactgcgcctcgttcctcggtgccagggacaccgtcgcgggaggcgcggccagcttccctaggataagacttcccgccccgggggcagggcggtgcacttagacggtcccctcctcagtttcgggcggtcaccagagctgagtaagctcggtggagggagctgggtaaggatttcctgagagcgatgggcaggaggggctggggcagcagagcacagagcaaggaccctgaacctgcgaacctgtccggcgacccgcgcgcctagcgccaccgcacgcgcgctctggcccccgggctacccgccctcgccggcccccgcccctccgggaggaagaagagggtaggtggggaggcggatgaggggtgggggaccccttgacgtcactggaaggaggtgccggggtaggaagtgggctggggaaaggttataaatcgcccccgccctcggctgcacttcagcgaggtccttgagaggctcggagcgcggtggcggacactcccgggaggtagtgctagtggtggtggctgctgctcggagcgggctccgggactcaagcgcagcggctagcggacgcgggacggcgaggatccccccacaccacccccctcggctgcaggcgcggagaagggctctcgcggcgccaagcagaagcaggaggggaccggctcgagcggctgcgccgtcggcctcggagagcgcgggc

SEQ ID NO: 10 - DNA, 423 bp, Artificial Sequence
  hEMCN
acattcactacaccttttccatttgctaataaggccctgccaggctgggagggaattgtccctgcctgcttctggagaaagaagatattgacaccatctacgggcaccatggaactgcttcaagtgaccattctttttcttctgcccagtatttgcagcagtaacagcacaggtatttttgtctcttattcctctggtggtacggattggaaatcactagtaggtgactcagcctcagtttactttcagggatcttcccctgacacttagatgcagcaattcctttgatgagttgagtgtttggatgttgacttggagtgcgtggagaaggcttgagagagacggtatttgtttctactgaagggaaatgtttgcgggtacagcagcctgaaagcatgttcgatgaaatcacaaagtactgga

SEQ ID NO: 11 - DNA, 738 bp, Artificial Sequence
  mEMCN
aggggaatgccagggccaagaagtgggagggggagggggagaggagtgggggggtatgggggacttttggaatagcagtggaaatgtaaatgaagaaaatatctaataaaaatatttaaaaagaaagaaagaaatgtcttgaaaacctctctgggcagtaataagaggccagcttacttcctcaagagcagaacgtgatccagttcatacttgtatttgcctctagaaggtggtcttcactgacttggcttatgagttgagaagagagaagaaatgcaattccttgtggattttgtactcaaatccagaccttgggaagtcacagccttttcagccgacctggggggctacttggtgaggtctctttacagcttctctaaaatgcactttcaaaacaaaagttagaaagctctctggccctttctcaagaagggtctcttcctgttcaaatcccatcctgacctttttgttgaagaagagtaaaataatgcagtaacaaaaacacaagtggctgccaaaggaagagagaggaaaaaaaaagaagttcctgtaaggggctgaaacaataaatctcctctctgctgacctcccaaagggagtgcgtgtatttcctctagttctttatcagaatccccaaaataagtaggaatgggcagcgtctgctcacagtcagtacacctttcccatttgctaatacggcctggccaggctgagaggaatccttccctgccttaccct

SEQ ID NO: 12 - DNA, 25 bp, Artificial Sequence
  attB1
acaagtttgtacaaaaaagcaggct

SEQ ID NO: 13 - DNA, 25 bp, Artificial Sequence
  attB2
accactttgtacaagaaagctgggt

SEQ ID NO: 14 - DNA, 588 bp, Artificial Sequence
  IRES
gcccctctccctcccccccccctaacgttactggccgaagccgcttggaataaggccggtgtgcgtttgtctatatgttattttccaccatattgccgtcttttggcaatgtgagggcccggaaacctggccctgtcttcttgacgagcattcctaggggtctttcccctctcgccaaaggaatgcaaggtctgttgaatgtcgtgaaggaagcagttcctctggaagcttcttgaagacaaacaacgtctgtagcgaccctttgcaggcagcggaaccccccacctggcgacaggtgcctctgcggccaaaagccacgtgtataagatacacctgcaaaggcggcacaaccccagtgccacgttgtgagttggatagttgtggaaagagtcaaatggctctcctcaagcgtattcaacaaggggctgaaggatgcccagaaggtaccccattgtatgggatctgatctggggcctcggtgcacatgctttacatgtgtttagtcgaggttaaaaaaacgtctaggccccccgaaccacggggacgtggttttcctttgaaaaacacgatgataatatggccacaacc

SEQ ID NO: 15 - DNA, 63 bp, Artificial Sequence
  T2A
ggaagcggagagggcaggggaagtcttctaacatgcggggacgtggaggaaaatcccggcccc

SEQ ID NO: 16 - DNA, 717 bp, Artificial Sequence
  eGFP
atggtgagcaagggcgaggagctgttcaccggggtggtgcccatcctggtcgagctggacggcgacgtaaacggccacaagttcagcgtgtccggcgagggcgagggcgatgccacctacggcaagctgaccctgaagttcatctgcaccaccggcaagctgcccgtgccctggcccaccctcgtgaccaccctgacctacggcgtgcagtgcttcagccgctaccccgaccacatgaagcagcacgacttcttcaagtccgccatgcccgaaggctacgtccaggagcgcaccatcttcttcaaggacgacggcaactacaagacccgcgccgaggtgaagttcgagggcgacaccctggtgaaccgcatcgagctgaagggcatcgacttcaaggaggacggcaacatcctggggcacaagctggagtacaactacaacagccacaacgtctatatcatggccgacaagcagaagaacggcatcaaggtgaacttcaagatccgccacaacatcgaggacggcagcgtgcagctcgccgaccactaccagcagaacacccccatcggcgacggccccgtgctgctgcccgacaaccactacctgagcacccagtccaagctgagcaaagaccccaacgagaagcgcgatcacatggtcctgctggagttcgtgaccgccgccgggatcactctcggcatggacgagctgtacaag

SEQ ID NO: 17 - DNA, 20 bp, Artificial Sequence
  hGAPDH Forward
cctccaaggagtaagacccc

SEQ ID NO: 18 - DNA, 20 bp, Artificial Sequence
  hGAPDH Reverse
aggggtctacatggcaactg

SEQ ID NO: 19 - DNA, 20 bp, Artificial Sequence
  hPLVAP Forward
agaactcagacctccaacgc

SEQ ID NO: 20 - DNA, 20 bp, Artificial Sequence
  hPLVAP Reverse
tctccaccttctgtttcgcc

SEQ ID NO: 21 - DNA, 19 bp, Artificial Sequence
  mGAPDH Forward
tgtccgtcgtggatctgac

SEQ ID NO: 22 - DNA, 20 bp, Artificial Sequence
  mGAPDH Reverse
cctgcttcaccaccttcttg

SEQ ID NO: 23 - DNA, 21 bp, Artificial Sequence
  mPLVAP Forward
gctggtactacctgcgctatt

SEQ ID NO: 24 - DNA, 20 bp, Artificial Sequence
  mPLVAP Reverse
cctgtgaggcagatagtcca

SEQ ID NO: 25 - protein, 442 aa, Artificial Sequence
  plasmalemma vesicle-associated protein [Homo sapiens]
MGLAMEHGGSYARAGGSSRGCWYYLRYFFLFVSLIQFLIILGLVLFMVYGNVHVSTESNLQATERRAEGLYSQLLGLTASQSNLTKELNFTTRAKDAIMQMWLNARRDLDRINASFRQCQGDRVIYTNNQRYMAAIILSEKQCRDQFKDMNKSCDALLFMLNQKVKTLEVEIAKEKTICTKDKESVLLNKRVAEEQLVECVKTRELQHQERQLAKEQLQKVQALCLPLDKDKFEMDLRNLWRDSIIPRSLDNLGYNLYHPLGSELASIRRACDHMPSLMSSKVEELARSLRADIERVARENSDLQRQKLEAQQGLRASQEAKQKVEKEAQAREAKLQAECSRQTQLALEEKAVLRKERDNLAKELEEKKREAEQLRMELAIRNSALDTCIKTKSQPMMPVSRPMGPVPNPQPIDPASLEEFKRKILESQRPPAGIPVAPSSG